European Patent Specification EP 3 636 776 B1, published October 9, 2024. Title: METHODS FOR DETECTING FETAL NUCLEIC ACIDS AND DIAGNOSING FETAL ABNORMALITIES. Applicant: SEQUENOM, INC. Application EP 11 745 050.2. The sequence listing filed with the application follows.

SEQUENCE LISTING (1 sequence)

SEQ ID NO: 1 - DNA, 32 bp, Artificial Sequence
  Synthetic oligonucleotide
tccacttatccttgcatccatcctctgccctg